European Patent Specification EP 3 757 231 B1, published April 1, 2026. Title: Primer set for detecting a gene of Trichophyton fungus by LAMP method, kit comprising it, and  method  for detecting the gene therewith. Applicant: SATO PHARMACEUTICAL CO., LTD Teikyo University. The sequence listing filed with the application follows.

SEQUENCE LISTING (32 sequences)

SEQ ID NO: 1 - DNA, 19 bp, Artificial Sequence
  Primer
aggatcattaacgcgcagg

SEQ ID NO: 2 - DNA, 19 bp, Artificial Sequence
  Primer
tcttggtgtctgtcctccg

SEQ ID NO: 3 - DNA, 38 bp, Artificial Sequence
  Primer
agaatgggggcgtacggccgatagggaccgacgttcca

SEQ ID NO: 4 - DNA, 39 bp, Artificial Sequence
  Primer
tctacctcacccggttgcctcgtcgaggctcccagaagg

SEQ ID NO: 5 - DNA, 18 bp, Artificial Sequence
  Primer
acgtctgctcacccctga

SEQ ID NO: 6 - DNA, 15 bp, Artificial Sequence
  Primer
ccgcgctccccctgc

SEQ ID NO: 7 - DNA, 19 bp, Artificial Sequence
  Primer
tgcggaaggatcattagcg

SEQ ID NO: 8 - DNA, 18 bp, Artificial Sequence
  Primer
ttttgcgtctgtcctccg

SEQ ID NO: 9 - DNA, 38 bp, Artificial Sequence
  Primer
caagaatggggcggtacggccccacgatagggccaaac

SEQ ID NO: 10 - DNA, 44 bp, Artificial Sequence
  Primer
tacattactcggttgcctcggcgcgtttagccactaaagagagg

SEQ ID NO: 11 - DNA, 20 bp, Artificial Sequence
  Primer
tctgctcacccctgacggac

SEQ ID NO: 12 - DNA, 17 bp, Artificial Sequence
  Primer
tctcccaggagagccgt

SEQ ID NO: 13 - DNA, 710 bp, Trichophyton rubrum
  ref <308>: GenBank U18352
  ref <309>: 1995-02-09
  ref <313>: (1)..(710)
aagtaaaagtcgtaacaaggtttccgtaggtgaacctgcggaaggatcattaacgcgcaggccggaggctggccccccacgatagggaccgacgttccatcaggggtgagcagacgtgcgccggccgtacgcccccattcttgtctacctcacccggttgcctcggcgggccgcgctccccctgccagggagagccgtccggcgggccccttctgggagcctcgagccggaccgcgcccgccggaggacagacaccaagaaaaaattctctgaagagctgtcagtctgagcgtttagcaagcacaatcagttaaaactttcaacaacggatctcttggttccggcatcgatgaagaacgcagcgaaatgcgataagtaatgtgaattgcagaattccgtgaatcatcgaatctttgaacgcacattgcgccctctggcattccggggggcatgcctgttcgagcgtcatttcaacccctcaagcccggcttgtgtgatggacgaccgtccggcccctcccttcgggggcgggacgcgcccgaaaagcagtggccaggccgcgattccggcttcctaggcgaatgggcagccaattcagcgccctcaggaccggccgccctggccccaatctttatatatatatatatcttttcaggttgacctcggatcaggtagggatacccgctgaacttaagcatatcaataagcgg

SEQ ID NO: 14 - DNA, 671 bp, Trichophyton mentagrophytes
  ref <308>: GenBank KC146353
  ref <309>: 2013-11-13
  ref <313>: (1)..(671)
ggtttccgtaggtgaacctgcggaaggatcattagcgcgcaggccggaggctggccccccacgatagggccaaacgtccgtcaggggtgagcagatgtgcgccggccgtaccgccccattcttgtctacattactcggttgcctcggcgggccgcgctctcccaggagagccgttcggcgagcctctctttagtggctaaacgctggaccgcgcccgccggaggacagacgcaaaaaaattctttcagaagagctgtcagtctgagcgttagcaagcaaaaatcagttaaaactttcaacaacggatctcttggttccggcatcgatgaagaacgcagcgaaatgcgataagtaatgtgaattgcagaattccgtgaatcatcgaatctttgaacgcacattgcgccccctggcattccggggggcatgcctgttcgagcgtcatttcagcccctcaagcccggcttgtgtgatggacgaccgtccggcgcccccgtctttgggggtgcgggacgcgcccgaaaagcagtggccaggccgcgattccggcttcctaggcgaatgggcaacaaaccagcgcctccaggaccggccgccctggcctcaaaatctgttttatacttatcaggttgacctcggatcaggtagggatacccgctgaacttaagcat

SEQ ID NO: 15 - DNA, 20 bp, Artificial Sequence
  Primer
aaggtttccgtaggtgaacc

SEQ ID NO: 16 - DNA, 17 bp, Artificial Sequence
  Primer
tcgaggctcccagaagg

SEQ ID NO: 17 - DNA, 41 bp, Artificial Sequence
  Primer
gaacgtcggtccctatcgtggtgcggaaggatcattaacgc

SEQ ID NO: 18 - DNA, 35 bp, Artificial Sequence
  Primer
ggccgtacgcccccattctacggctctccctggca

SEQ ID NO: 19 - DNA, 19 bp, Artificial Sequence
  Primer
tctacctcacccggttgcc

SEQ ID NO: 20 - DNA, 15 bp, Artificial Sequence
  Primer
cagcctccggcctgc

SEQ ID NO: 21 - DNA, 19 bp, Artificial Sequence
  Priemr
tgaacctgcggaaggatca

SEQ ID NO: 22 - DNA, 19 bp, Artificial Sequence
  Primer
tcttggtgtctgtcctccg

SEQ ID NO: 23 - DNA, 35 bp, Artificial Sequence
  Primer
agaatgggggcgtacggcctggccccccacgatag

SEQ ID NO: 24 - DNA, 39 bp, Artificial Sequence; identical to SEQ ID NO: 4
  Primer

SEQ ID NO: 25 - DNA, 18 bp, Artificial Sequence
  Primer
ccacgatagggccaaacg

SEQ ID NO: 26 - DNA, 21 bp, Artificial Sequence
  Primer
ctcagactgacagctcttctg

SEQ ID NO: 27 - DNA, 40 bp, Artificial Sequence
  Primer
gccgaggcaaccgagtaatgtacgtcaggggtgagcagat

SEQ ID NO: 28 - DNA, 42 bp, Artificial Sequence
  Primer
cgttcggcgagcctctctttaatttttttgcgtctgtcctcc

SEQ ID NO: 29 - DNA, 19 bp, Artificial Sequence
  Primer
tcaggggtgagcagatgtg

SEQ ID NO: 30 - DNA, 20 bp, Artificial Sequence
  Primer
gctcagactgacagctcttc

SEQ ID NO: 31 - DNA, 38 bp, Artificial Sequence
  Primer
aacggctctcctgggagagccgtaccgccccattcttg

SEQ ID NO: 32 - DNA, 43 bp, Artificial Sequence
  Primer
cggcgagcctctctttagtggaatttttttgcgtctgtcctcc